European Patent Application EP 4 286 010 A1, published December 6, 2023. Title: ANTI-CD20 ANTIBODY COMPOSITIONS. Applicant: TG Therapeutics, Inc. Application EP. The sequence listing filed with the application follows.

SEQUENCE LISTING (38 sequences)

SEQ ID NO: 1 - protein, 448 aa, synthetic construct
QAYLQQSGAELVRPGASVKMSCKASGYTFTSYNMHWVKQTPRQGLEWIGGIYPGNGDTSYNQKFKGKATLTVGKSSSTAYMQLSSLTSEDSAVYFCARYDYNYAMDYWGQGTSVTVSSASTKGPSVFPLAPSSKSTSGGTAALGCLVKDYFPEPVTVSWNSGALTSGVHTFPAVLQSSGLYSLSSVVTVPSSSLGTQTYICNVNHKPSNTKVDKKVEPKSCDKTHTCPPCPAPELLGGPSVFLFPPKPKDTLMISRTPEVTCVVVDVSHEDPEVKFNWYVDGVEVHNAKTKPREEQYNSTYRVVSVLTVLHQDWLNGKEYKCKVSNKALPAPIEKTISKAKGQPREPQVYTLPPSRDELTKNQVSLTCLVKGFYPSDIAVEWESNGQPENNYKTTPPVLDSDGSFFLYSKLTVDKSRWQQGNVFSCSVMHEALHNHYTQKSLSLSPGK

SEQ ID NO: 2 - protein, 213 aa, synthetic construct
QIVLSQSPAILSASPGEKVTMTCRASSSVSYMHWYQQKPGSSPKPWIYATSNLASGVPARFSGSGSGTSYSFTISRVEAEDAATYYCQQWTFNPPTFGGGTRLEIKRTVAAPSVFIFPPSDEQLKSGTASVVCLLNNFYPREAKVQWKVDNALQSGNSQESVTEQDSKDSTYSLSSTLTLSKADYEKHKVYACEVTHQGLSSPVTKSFNRGEC

SEQ ID NO: 3 - protein, 7 aa, synthetic construct
GYTFTSY

SEQ ID NO: 4 - protein, 6 aa, synthetic construct
YPGNGD

SEQ ID NO: 5 - protein, 9 aa, synthetic construct
YDYNYAMDY

SEQ ID NO: 6 - protein, 118 aa, synthetic construct
QAYLQQSGAELVRPGASVKMSCKASGYTFTSYNMHWVKQTPRQGLEWIGGIYPGNGDTSYNQKFKGKATLTVGKSSSTAYMQLSSLTSEDSAVYFCARYDYNYAMDYWGQGTSVTVSS

SEQ ID NO: 7 - protein, 330 aa, synthetic construct [sequence omitted]

SEQ ID NO: 8 - protein, 10 aa, synthetic construct
RASSSVSYMH

SEQ ID NO: 9 - protein, 7 aa, synthetic construct
ATSNLAS

SEQ ID NO: 10 - protein, 9 aa, synthetic construct
QQWTFNPPT

SEQ ID NO: 11 - protein, 107 aa, synthetic construct
QIVLSQSPAILSASPGEKVTMTCRASSSVSYMHWYQQKPGSSPKPWIYATSNLASGVPARFSGSGSGTSYSFTISRVEAEDAATYYCQQWTFNPPTFGGGTRLEIKR

SEQ ID NO: 12 - protein, 106 aa, synthetic construct
TVAAPSVFIFPPSDEQLKSGTASVVCLLNNFYPREAKVQWKVDNALQSGNSQESVTEQDSKDSTYSLSSTLTLSKADYEKHKVYACEVTHQGLSSPVTKSFNRGEC

SEQ ID NO: 13 - protein, 448 aa, synthetic construct
  source 1..448: note = Modified heavy chain (substitution of glutamine at position 1 with pyroglutamate)
EAYLQQSGAELVRPGASVKMSCKASGYTFTSYNMHWVKQTPRQGLEWIGGIYPGNGDTSYNQKFKGKATLTVGKSSSTAYMQLSSLTSEDSAVYFCARYDYNYAMDYWGQGTSVTVSSASTKGPSVFPLAPSSKSTSGGTAALGCLVKDYFPEPVTVSWNSGALTSGVHTFPAVLQSSGLYSLSSVVTVPSSSLGTQTYICNVNHKPSNTKVDKKVEPKSCDKTHTCPPCPAPELLGGPSVFLFPPKPKDTLMISRTPEVTCVVVDVSHEDPEVKFNWYVDGVEVHNAKTKPREEQYNSTYRVVSVLTVLHQDWLNGKEYKCKVSNKALPAPIEKTISKAKGQPREPQVYTLPPSRDELTKNQVSLTCLVKGFYPSDIAVEWESNGQPENNYKTTPPVLDSDGSFFLYSKLTVDKSRWQQGNVFSCSVMHEALHNHYTQKSLSLSPGK

SEQ ID NO: 14 - protein, 213 aa, synthetic construct
  source 1..213: note = Modified light chain (substitution of glutamine at position 1 with pyroglutamate)
EIVLSQSPAILSASPGEKVTMTCRASSSVSYMHWYQQKPGSSPKPWIYATSNLASGVPARFSGSGSGTSYSFTISRVEAEDAATYYCQQWTFNPPTFGGGTRLEIKRTVAAPSVFIFPPSDEQLKSGTASVVCLLNNFYPREAKVQWKVDNALQSGNSQESVTEQDSKDSTYSLSSTLTLSKADYEKHKVYACEVTHQGLSSPVTKSFNRGEC

SEQ ID NO: 15 - protein, 447 aa, synthetic construct
QAYLQQSGAELVRPGASVKMSCKASGYTFTSYNMHWVKQTPRQGLEWIGGIYPGNGDTSYNQKFKGKATLTVGKSSSTAYMQLSSLTSEDSAVYFCARYDYNYAMDYWGQGTSVTVSSASTKGPSVFPLAPSSKSTSGGTAALGCLVKDYFPEPVTVSWNSGALTSGVHTFPAVLQSSGLYSLSSVVTVPSSSLGTQTYICNVNHKPSNTKVDKKVEPKSCDKTHTCPPCPAPELLGGPSVFLFPPKPKDTLMISRTPEVTCVVVDVSHEDPEVKFNWYVDGVEVHNAKTKPREEQYNSTYRVVSVLTVLHQDWLNGKEYKCKVSNKALPAPIEKTISKAKGQPREPQVYTLPPSRDELTKNQVSLTCLVKGFYPSDIAVEWESNGQPENNYKTTPPVLDSDGSFFLYSKLTVDKSRWQQGNVFSCSVMHEALHNHYTQKSLSLSPG

SEQ ID NO: 16 - protein, 213 aa, synthetic construct
QIVLSQSPAILSASPGEKVTMTCRASSSVSYMHWYQQKPGSSPKPWIYATSNLASGVPARFSGSGSGTSYSFTISRVEAEDAATYYCQQWTFNPPTFGGGTRLEINRTVAAPSVFIFPPSDEQLKSGTASVVCLLNNFYPREAKVQWKVDNALQSGNSQESVTEQDSKDSTYSLSSTLTLSKADYEKHKVYACEVTHQGLSSPVTKSFNRGEC

SEQ ID NO: 17 - protein, 4 aa, synthetic construct
MSCK

SEQ ID NO: 18 - protein, 15 aa, synthetic construct
ASGYTFTSYNMHWVK

SEQ ID NO: 19 - protein, 25 aa, synthetic construct
QTPRQGLEWIGGIYPGNGDTSYNQK

SEQ ID NO: 20 - protein, 9 aa, synthetic construct
GKATLTVGK

SEQ ID NO: 21 - protein, 48 aa, synthetic construct
SSSTAYMQLSSLTSEDSAVYFCARYDYNYAMDYWGQGTSVTVSSASTK

SEQ ID NO: 22 - protein, 58 aa, synthetic construct
DYFPEPVTVSWNSGALTSGVHTFPAVLQSSGLYSLSSVVTVPSSSLGTQTYICNVNHK

SEQ ID NO: 23 - protein, 28 aa, synthetic construct
PKDTLMISRTPEVTCVVVDVSHEDPEVK

SEQ ID NO: 24 - protein, 26 aa, synthetic construct
DTLMISRTPEVTCVVVDVSHEDPEVK

SEQ ID NO: 25 - protein, 14 aa, synthetic construct
FNWYVDGVEVHNAK

SEQ ID NO: 26 - protein, 12 aa, synthetic construct
VSNKALPAPIEK

SEQ ID NO: 27 - protein, 10 aa, synthetic construct
NQVSLTCLVK

SEQ ID NO: 28 - protein, 22 aa, synthetic construct
GFYPSDIAVEWESNGQPENNYK

SEQ ID NO: 29 - protein, 25 aa, synthetic construct
SRWQQGNVFSCSVMHEALHNHYTQK

SEQ ID NO: 30 - protein, 20 aa, synthetic construct
VTMTCRASSSVSYMHWYQQK

SEQ ID NO: 31 - protein, 19 aa, synthetic construct
SGTASVVCLLNNFYPREAK

SEQ ID NO: 32 - protein, 20 aa, synthetic construct
VDNALQSGNSQESVTEQDSK

SEQ ID NO: 33 - protein, 29 aa, synthetic construct
TKPREEQYNSTYRVVSVLTVLHQDWLNGK

SEQ ID NO: 34 - protein, 23 aa, synthetic construct
DIAVEWESNGQPENNYKTTPPVL

SEQ ID NO: 35 - DNA, 1344 bp, synthetic construct
  source 1..1344: mol_type = other DNA
caggcttatctacagcagtctggggctgagctggtgaggcctggggcctcagtgaagatgtcctgcaaggcttctggctacacatttaccagttacaatatgcactgggtaaagcagacacctagacagggcctggaatggattggaggtatttatccaggaaatggtgatacttcctacaatcagaagttcaagggcaaggccacactgactgtaggcaaatcctccagcacagcctacatgcagctcagcagcctgacatctgaagactctgcggtctatttctgtgcaagatatgactacaactatgctatggactactggggtcaaggaacctcagtcaccgtctcctcagcctccaccaagggcccatcggtcttccccctggcaccctcctccaagagcacctctgggggcacagcggccctgggctgcctggtcaaggactacttccccgaaccggtgacggtgtcgtggaactcaggcgccctgaccagcggcgtgcacaccttcccggctgtcctacagtcctcaggactctactccctcagcagcgtggtgaccgtgccctccagcagcttgggcacccagacctacatctgcaacgtgaatcacaagcccagcaacaccaaggtggacaagaaagttgagcccaaatcttgtgacaaaactcacacatgcccaccgtgcccagcacctgaactcctggggggaccgtcagtcttcctcttccccccaaaacccaaggacaccctcatgatctcccggacccctgaggtcacatgcgtggtggtggacgtgagccacgaagaccctgaggtcaagttcaactggtacgtggacggcgtggaggtgcataatgccaagacaaagccgcgggaggagcagtacaacagcacgtaccgtgtggtcagcgtcctcaccgtcctgcaccaggactggctgaatggcaaggagtacaagtgcaaggtctccaacaaagccctcccagcccccatcgagaaaaccatctccaaagccaaagggcagccccgagaaccacaggtgtacaccctgcccccatcccgggatgagctgaccaagaaccaggtcagcctgacctgcctggtcaaaggcttctatcccagcgacatcgccgtggagtgggagagcaatgggcagccggagaacaactacaagaccacgcctcccgtgctggactccgacggctccttcttcctctacagcaagctcaccgtggacaagagcaggtggcagcaggggaacgtcttctcatgctccgtgatgcatgaggctctgcacaaccactacacgcagaagagcctctccctgtctccgggtaaa

SEQ ID NO: 36 - DNA, 639 bp, synthetic construct
  source 1..639: mol_type = other DNA
caaattgttctctcccagtctccagcaatcctgtctgcatctccaggggagaaggtcacaatgacttgcagggccagctcaagtgtaagttacatgcactggtaccagcagaagccaggatcctcccccaaaccctggatttatgccacatccaacctggcttctggagtccctgctcgcttcagtggcagtgggtctgggacctcttattctttcacaatcagcagagtggaggctgaagatgctgccacttattactgccagcagtggacttttaacccacccacgttcggaggggggaccaggctggaaataaaacggactgtggctgcaccaagtgtcttcatcttcccgccatctgatgagcagttgaaatctggaactgcctctgttgtgtgcctgctgaataacttctatcccagagaggccaaagtacagtggaaggtggataacgccctccaatcgggtaactcccaggagagtgtcacagagcaggacagcaaggacagcacctacagcctcagcagcaccctgacgctgagcaaagcagactacgagaaacacaaagtctacgcctgcgaagtcacccatcagggcctgagctcgcccgtcacaaagagcttcaacaggggagagtgt

SEQ ID NO: 37 - protein, 5 aa, synthetic construct
IRAHT

SEQ ID NO: 38 - protein, 4 aa, synthetic construct
EPAN